European Patent Application EP 4 406 967 A1, published July 31, 2024. Title: RECOMBINANT THYROID-STIMULATING HORMONE RECEPTOR PROTEIN, PREPARATION METHOD AND APPLICATION THEREOF. Applicant: XIAMEN INNOBIOMAX BIOTECHNOLOGY CO., LTD. XIAMEN INNODX BIOTECH CO., LTD. The sequence listing filed with the application follows.

SEQUENCE LISTING (13 sequences)

SEQ ID NO: 1 - DNA, 2295 bp, Artificial sequence
  cDNA sequence of human TSHR (hTSHR)
atgaggccggcggacttgctgcagctggtgctgctgctcgacctgcccagggacctgggcggaatggggtgttcgtctccaccctgcgagtgccatcaggaggaggacttcagagtcacctgcaaggatattcaacgcatccccagcttaccgcccagtacgcagactctgaagcttattgagactcacctgagaactattccaagtcatgcattttctaatctgcccaatatttccagaatctacgtatctatagatgtgactctgcagcagctggaatcacactccttctacaatttgagtaaagtgactcacatagaaattcggaataccaggaacttaacttacatagaccctgatgccctcaaagagctccccctcctaaagttccttggcattttcaacactggacttaaaatgttccctgacctgaccaaagtttattccactgatatattctttatacttgaaattacagacaacccttacatgacgtcaatccctgtgaatgcttttcagggactatgcaatgaaaccttgacactgaagctgtacaacaatggctttacttcagtccaaggatatgctttcaatgggacaaagctggatgctgtttacctaaacaagaataaatacctgacagttattgacaaagatgcatttggaggagtatacagtggaccaagcttgctggacgtgtctcaaaccagtgtcactgcccttccatccaaaggcctggagcacctgaaggaactgatagcaagaaacacctggactcttaagaaacttccactttccttgagtttccttcacctcacacgggctgacctttcttacccaagccactgctgtgcttttaagaatcagaagaaaatcagaggaatccttgagtccttgatgtgtaatgagagcagtatgcagagcttgcgccagagaaaatctgtgaatgccttgaatagccccctccaccaggaatatgaagagaatctgggtgacagcattgttgggtacaaggaaaagtccaagttccaggatactcataacaacgctcattattacgtcttctttgaagaacaagaggatgagatcattggttttggccaggagctcaaaaacccccaggaagagactctacaagcttttgacagccattatgactacaccatatgtggggacagtgaagacatggtgtgtacccccaagtccgatgagttcaacccgtgtgaagacataatgggctacaagttcctgagaattgtggtgtggttcgttagtctgctggctctcctgggcaatgtctttgtcctgcttattctcctcaccagccactacaaactgaacgtcccccgctttctcatgtgcaacctggcctttgcggatttctgcatggggatgtacctgctcctcatcgcctctgtagacctctacactcactctgagtactacaaccatgccatcgactggcagacaggccctgggtgcaacacggctggtttcttcactgtctttgcaagcgagttatcggtgtatacgctgacggtcatcaccctggagcgctggtatgccatcaccttcgccatgcgcctggaccggaagatccgcctcaggcacgcatgtgccatcatggttgggggctgggtttgctgcttccttctcgccctgcttcctttggtgggaataagtagctatgccaaagtcagtatctgcctgcccatggacaccgagacccctcttgctctggcatatattgtttttgttctgacgctcaacatagttgccttcgtcatcgtctgctgctgttatgtgaagatctacatcacagtccgaaatccgcagtacaacccaggggacaaagataccaaaattgccaagaggatggctgtgttgatcttcaccgacttcatatgcatggccccaatctcattctatgctctgtcagcaattctgaacaagcctctcatcactgttagcaactccaaaatcttgctggtactcttctatccacttaactcctgtgccaatccattcctctatgctattttcaccaaggccttccagagggatgtgttcatcctactcagcaagtttggcatctgtaaacgccaggctcaggcataccgggggcagagggttcctccaaagaacagcactgatattcaggttcaaaaggttacccacgagatgaggcagggtctccacaacatggaagatgtctatgaactgattgaaaactcccatctaaccccaaagaagcaaggccaaatctcagaagagtatatgcaaacggttttgtaa

SEQ ID NO: 2 - DNA, 681 bp, Artificial sequence
  cDNA sequence of human antibody IgG1
gacaaaactcacacatgcccaccgtgcccagcacctgaactcctggggggaccgttagtcttcctcttccccccaaaacccaaggacaccctcatgatctcccggacccctgaggtcacatgcgtggtggtggacgtgagccacgaagaccctgaggtcaagttcaactggtacgtggacggcgtggaggtgcataatgccaagacaaagccgcgggaggagcagtacaacagcacgtaccgtgtggtcagcgtcctcaccgtcctgcaccaggactggctgaatggcaaggagtacaagtgcaaggtctccaacaaagccctcccagcccccatcgagaaaaccatctccaaagccaaagggcagccccgagaaccacaggtgtacaccctgcccccatcccgggacgagctgaccaagaaccaggtcagcctgacctgcctggtcaaaggcttctatcccagcgacatcgccgtggagtgggagagcaatgggcagccggagaacaactacaagaccacgcctcccgtgctggactccgacggctccttcttcctctacagcaagctcaccgtggacaagagcaggtggcagcaggggaacgtcttctcatgctccgtgatgcatgaggctctgcacaaccactacacgcagaagagcctctccctgtctccgggtaaa

SEQ ID NO: 3 - DNA, 48 bp, Artificial sequence
  upstream primer sequence PF1
tctgcctttgcggcggatcttggatccatgggctgcagcagtccgccg

SEQ ID NO: 4 - DNA, 42 bp, Artificial sequence
  upstream primer sequence PF2
gatattatgggttataaatttgcaatttttaccaaagccttt

SEQ ID NO: 5 - DNA, 48 bp, Artificial sequence
  upstream primer sequence PF3
gaatatatgcagaccgttctggaattcgacaaaactcacacatgccca

SEQ ID NO: 6 - DNA, 33 bp, Artificial sequence
  downstream primer sequence PR1
aaatttataacccataatatcttcacacggatt

SEQ ID NO: 7 - DNA, 30 bp, Artificial sequence
  downstream primer sequence PR2
gaattccagaacggtctgcatatattcttc

SEQ ID NO: 8 - DNA, 57 bp, Artificial sequence
  downstream primer sequence PR3
gtcccaggaaaggatcagatctgcagcggccgcttatttacccggagacagggagag

SEQ ID NO: 9 - DNA, 1185 bp, Artificial sequence
  codon-optimized nucleotide sequence of hTSHR 64-1248 bp
atgggctgcagcagtccgccgtgtgaatgtcatcaggaagaagattttcgtgtgacctgtaaagatattcagcgtattccgagcctgccgccgagcacccagaccttaaaactgattgaaacccatctgcgtaccattccgagtcatgcattttctaatctgccgaatattagccgcatctatgttagcattgatgttaccctgcagcagctggaaagccatagcttttataatctgagcaaagtgacccatattgaaattcgcaatacccgtaatctgacctatattgatccggatgcactgaaagaactgccgctgctgaaatttctgggcatttttaataccggtctgaaaatgtttccggatctgaccaaagtttatagtaccgatattttctttatcctggaaattaccgataacccgtatatgaccagcattccggtgaatgcctttcagggtctgtgcaatgaaaccctgaccctgaaactgtataataatggttttaccagtgtgcagggctatgcctttaatggcaccaaactggatgccgtgtatctgaataagaataagtatctgaccgtgattgataaagatgcctttggcggcgtgtatagcggtccgagtctgctggatgttagtcagaccagtgttaccgcactgccgagcaaaggtctggaacatctgaaagaattaattgcacgtaatacctggaccctgaaaaaactgccgctgagcctgagctttctgcatctgacccgtgccgatctgagttatccgagccattgttgtgcctttaaaaatcagaaaaagatccgtggtatcctggaaagtctgatgtgcaatgaaagcagcatgcagagcctgcgtcagcgcaaaagcgtgaatgcactgaatagcccgctgcatcaggaatatgaagaaaatctgggcgatagtattgtgggctataaagaaaaaagtaagttccaggatacccataataatgcccattattatgttttcttcgaggaacaggaagatgaaattattggttttggtcaggaactgaaaaatccgcaggaagaaaccctgcaggcctttgatagccattatgattataccatttgcggcgatagtgaagatatggtgtgcaccccgaaaagtgatgagtttaatccgtgtgaagatattatgggttataaattt

SEQ ID NO: 10 - DNA, 258 bp, Artificial sequence
  codon-optimized nucleotide sequence of hTSHR 2035-2292 bp
gcaatttttaccaaagcctttcagcgtgatgtttttattctgctgagtaaatttggtatctgtaaacgccaggcccaggcatatcgtggccagcgcgttccgccgaaaaatagcaccgatattcaggtgcagaaagttacccatgaaatgcgtcagggtctgcataatatggaagatgtgtatgaactgattgaaaatagtcatctgaccccgaaaaaacagggccagattagcgaagaatatatgcagaccgttctg

SEQ ID NO: 11 - protein, 764 aa, Artificial sequence
  amino acid sequence of human TSHR (hTSHR)
MRPADLLQLVLLLDLPRDLGGMGCSSPPCECHQEEDFRVTCKDIQRIPSLPPSTQTLKLIETHLRTIPSHAFSNLPNISRIYVSIDVTLQQLESHSFYNLSKVTHIEIRNTRNLTYIDPDALKELPLLKFLGIFNTGLKMFPDLTKVYSTDIFFILEITDNPYMTSIPVNAFQGLCNETLTLKLYNNGFTSVQGYAFNGTKLDAVYLNKNKYLTVIDKDAFGGVYSGPSLLDVSQTSVTALPSKGLEHLKELIARNTWTLKKLPLSLSFLHLTRADLSYPSHCCAFKNQKKIRGILESLMCNESSMQSLRQRKSVNALNSPLHQEYEENLGDSIVGYKEKSKFQDTHNNAHYYVFFEEQEDEIIGFGQELKNPQEETLQAFDSHYDYTICGDSEDMVCTPKSDEFNPCEDIMGYKFLRIVVWFVSLLALLGNVFVLLILLTSHYKLNVPRFLMCNLAFADFCMGMYLLLIASVDLYTHSEYYNHAIDWQTGPGCNTAGFFTVFASELSVYTLTVITLERWYAITFAMRLDRKIRLRHACAIMVGGWVCCFLLALLPLVGISSYAKVSICLPMDTETPLALAYIVFVLTLNIVAFVIVCCCYVKIYITVRNPQYNPGDKDTKIAKRMAVLIFTDFICMAPISFYALSAILNKPLITVSNSKILLVLFYPLNSCANPFLYAIFTKAFQRDVFILLSKFGICKRQAQAYRGQRVPPKNSTDIQVQKVTHEMRQGLHNMEDVYELIENSHLTPKKQGQISEEYMQTVL

SEQ ID NO: 12 - protein, 395 aa, Artificial sequence
  amino acid sequence of extracellular segment of hTSHR
MGCSSPPCECHQEEDFRVTCKDIQRIPSLPPSTQTLKLIETHLRTIPSHAFSNLPNISRIYVSIDVTLQQLESHSFYNLSKVTHIEIRNTRNLTYIDPDALKELPLLKFLGIFNTGLKMFPDLTKVYSTDIFFILEITDNPYMTSIPVNAFQGLCNETLTLKLYNNGFTSVQGYAFNGTKLDAVYLNKNKYLTVIDKDAFGGVYSGPSLLDVSQTSVTALPSKGLEHLKELIARNTWTLKKLPLSLSFLHLTRADLSYPSHCCAFKNQKKIRGILESLMCNESSMQSLRQRKSVNALNSPLHQEYEENLGDSIVGYKEKSKFQDTHNNAHYYVFFEEQEDEIIGFGQELKNPQEETLQAFDSHYDYTICGDSEDMVCTPKSDEFNPCEDIMGYKF

SEQ ID NO: 13 - protein, 86 aa, Artificial sequence
  amino acid sequence of intracellular segment of hTSHR
AIFTKAFQRDVFILLSKFGICKRQAQAYRGQRVPPKNSTDIQVQKVTHEMRQGLHNMEDVYELIENSHLTPKKQGQISEEYMQTVL